European Patent Application EP 4 122 958 A1, published January 25, 2023. Title: Anti-ROR2 Antibodies. Applicant: BioAtla Inc. The sequence listing filed with the application follows.

SEQUENCE LISTING (27 sequences)

SEQ ID NO: 1 - protein, 10 aa, Artificial Sequence
  Synthetic sequence
  misc_feature (4)..(4): Xaa can be any naturally occurring amino acid
  misc_feature (7)..(7): Xaa can be any naturally occurring amino acid
  misc_feature (9)..(9): Xaa can be any naturally occurring amino acid
GYTXTEXTXH

SEQ ID NO: 2 - protein, 17 aa, Artificial Sequence
  Synthetic sequence
  misc_feature (2)..(2): Xaa can be any naturally occurring amino acid
  misc_feature (4)..(4): Xaa can be any naturally occurring amino acid
GXNXNNGGTGYNQKFKG

SEQ ID NO: 3 - protein, 13 aa, Artificial Sequence
  Synthetic sequence
GSLYSYGNSYFDY

SEQ ID NO: 4 - protein, 12 aa, Artificial
  Synthetic sequence
  misc_feature (1)..(1): Xaa can be any naturally occurring amino acid
  misc_feature (9)..(9): Xaa can be any naturally occurring amino acid
XGYSITTGXYWN

SEQ ID NO: 5 - protein, 16 aa, Artificial
  Synthetic sequence
YITYDGSKNYNPSLKN

SEQ ID NO: 6 - protein, 10 aa, Artificial
  Synthetic sequence
  misc_feature (6)..(6): Xaa can be any naturally occurring amino acid
FEGVWXGLDY

SEQ ID NO: 7 - protein, 10 aa, Artificial Sequence
  Synthetic sequence
  misc_feature (6)..(6): Xaa can be any naturally occurring amino acid
SATSSXSYMH

SEQ ID NO: 8 - protein, 7 aa, Artificial Sequence
  Synthetic sequence
  misc_feature (1)..(1): Xaa can be any naturally occurring amino acid
XTSNLAS

SEQ ID NO: 9 - protein, 9 aa, Artificial Sequence
  Synthetic sequence
QQRSSYPFT

SEQ ID NO: 10 - protein, 15 aa, Artificial
  Synthetic sequence
RASESVDRYGNSFIH

SEQ ID NO: 11 - protein, 7 aa, Artificial
  Synthetic sequence
RTYNLES

SEQ ID NO: 12 - protein, 9 aa, Artificial
  Synthetic sequence
QQTNEDPWT

SEQ ID NO: 13 - protein, 106 aa, Artificial
  Synthetic sequence
QIVLTQSPAIMSASPGEKVTITCSATSSVSYMHWFQQKPGTSPKLWIYGTSNLASGVPARFSGSGSGTSYSLTISRMEAEDAATYYCQQRSSYPFTFGQGTKVEIK

SEQ ID NO: 14 - protein, 106 aa, Artificial
  Synthetic sequence
QIVLTQSPAIMSASPGEKVTITCSATSSESYMHWFQQKPGTSPKLWIYHTSNLASGVPARFSGSGSGTSYSLTISRMEAEDAATYYCQQRSSYPFTFGQGTKVEIK

SEQ ID NO: 15 - protein, 106 aa, Artificial
  Synthetic sequences
AIQLTQSPSSLSASVGDRVTITCSATSSVSYMHWYQQKPGQAPRLLIYGTSNLASGVPDRFSGSGSGTDFTLKISRVEAEDVGVYYCQQRSSYPFTFGQGTKVEIK

SEQ ID NO: 16 - protein, 106 aa, Artificial
  Synthetic sequence
AIQLTQSPSSLSASVGDRVTITCSATSSVSYMHWYLQKPGQSPQLLIYGTSNLASGVPDRFSGSGSGTDFTLKISRVEAEDVGVYYCQQRSSYPFTFGQGTKVEIK

SEQ ID NO: 17 - protein, 111 aa, Artificial
  Synthetic sequence
DIVLTQSPDSLAVSLGQRATISCRASESVDRYGNSFIHWYLQKPGQPPKLLIYRTYNLESGIPARFSGTGSRTDFTLTINPVEADDVATYYCQQTNEDPWTFGQGTKVEIK

SEQ ID NO: 18 - protein, 122 aa, Artificial
  Synthetic sequence
EVQLQQSGPELVKPGASVKISCKTSGYTFTEYTMHWMKQSHRKSLEWIGGINTNNGGTGYNQKFKGKATLTVDKSSSTAYMELRSLTSEDSAVYFCARGSLYSYGNSYFDYWGQGTLVTVSS

SEQ ID NO: 19 - protein, 122 aa, Artificial
  Synthetic sequence
EVQLQQSGPELVKPGASVKISCKTSGYTETEDTDHWMKQSHRKSLEWIGGENDNNGGTGYNQKFKGKATLTVDKSSSTAYMELRSLTSEDSAVYFCAHGSLYSYGNSYFDYWGQGTLVTVSS

SEQ ID NO: 20 - protein, 122 aa, Artificial
  Synthetic sequence
QVQLVQSGAEVKKPGASVKVSCKASGYTFTEYTMHWVRQARGQRLEWIGGINTNNGGTGYNQKFKGRVTISADKSISTAYLQWSSLKASDTAMYYCAHGSLYSYGNSYFDYWGQGTLVTVSS

SEQ ID NO: 21 - protein, 122 aa, Artificial
  Synthetic sequence
EVQLVQSGAEVKKPGESLRISCKGSGYTFTEYTMHWVRQAPGQGLEWMGGINTNNGGTGYNQKFKGRVTISADKSISTAYLQWSSLKASDTAMYYCAHGSLYSYGNSYFDYWGQGTLVTVSS

SEQ ID NO: 22 - protein, 122 aa, Artificial
  Synthetic sequence
EVQLVQSGAEVKKPGESLRISCKGSGYTFTEYTMHWIRQSPSRGLEWLGGINTNNGGTGYNQKFKGRVTISADKSISTAYLQWSSLKASDTAMYYCAHGSLYSYGNSYFDYWGQGTLVTVSS

SEQ ID NO: 23 - protein, 119 aa, Artificial
  Synthetic sequence
DVQLQESGPGLVKPSQSLSLTCSVTGYSITTGYYWNWIRQFPGNKLEWMAYITYDGSKNYNPSLKNRISITRDTSKNKFFLKLNSVTSEDTATYYCSRFEGVWYGLDYWGQGTLVTVSS

SEQ ID NO: 24 - protein, 119 aa, Artificial
  Synthetic sequence
DVQLQESGPGLVKPSQSLSLTCSVTGYSITTGYYWNWIRQFPGNKLEWMAYITYDGSKNYNPSLKNRISITRDTSKNKFFLKLNSVTSEDTATYYCSHFEGVWGGLDYWGQGTLVTVSS

SEQ ID NO: 25 - protein, 119 aa, Artificial
  Synthetic sequence
QVQLQESGPGLVKPSQTLSLTCTVSGYSITTGYYWNWVRQARGQRLEWIGYITYDGSKNYNPSLKNRVTISVDTSKNQFSLKLSSVTAADTAVYYCSHFEGVWYGLDYWGQGTLVTVSS

SEQ ID NO: 26 - protein, 119 aa, Artificial sequence
  Synthetic sequence
QVQLQESGPGLVKPSQTLSLTCTVSGYSITTGEYWNWVRQARGQRLEWIGYITYDGSKNYNPSLKNRVTISVDTSKNQFSLKLSSVTAADTAVYYCSRFEGVWYGLDYWGQGTLVTVSS

SEQ ID NO: 27 - protein, 111 aa, Artificial
  Synthetic sequence
AIQLTQSPSSLSASVGDRVTITCRASESVDRYGNSFIHWYQQKPGKAPKLLIYRTYNLESGIPARFSGSGSGTEFTLTISSLQSEDFAVYYCQQTNEDPWTFGQGTKVEIK